European Patent Specification EP 3 574 008 B1, published November 8, 2023. Title: Hemagglutinin-Specific Antibodies and Uses Thereof. Applicant: National Research Council of Canada. The sequence listing filed with the application follows.

SEQUENCE LISTING (36 sequences)

SEQ ID NO: 1 - protein, 12 aa, Artificial Sequence
  Complementarity determining region (CDR) L1 sequence
  MISC_FEATURE (7)..(7): Wherein X is R or D
  MISC_FEATURE (8)..(8): Wherein X is N or T
  MISC_FEATURE (12)..(12): Wherein X is H or F
QSLLNSXXQKNX

SEQ ID NO: 2 - protein, 9 aa, Artificial Sequence
  Complementarity determining region (CDR) L3 sequence
  MISC_FEATURE (5)..(5): Wherein X is T or S
  MISC_FEATURE (6)..(6): Wherein X is Y or I
  MISC_FEATURE (7)..(7): Wherein X is P or no amino acid
  MISC_FEATURE (8)..(8): Wherein X is R or L
QQYYXXXXT

SEQ ID NO: 3 - protein, 9 aa, Artificial Sequence
  Complementarity determining region (CDR) H1 sequence
  MISC_FEATURE (3)..(3): Wherein X is S or T
  MISC_FEATURE (4)..(4): Wherein X is I or F
  MISC_FEATURE (6)..(6): Wherein X is S or no amino acid
GYXXTXDYY

SEQ ID NO: 4 - protein, 7 aa, Artificial Sequence
  Complementarity determining region (CDR) H2 sequence
  MISC_FEATURE (6)..(6): Wherein X is S or T
IGYDGXK

SEQ ID NO: 5 - protein, 8 aa, Artificial Sequence
  Complementarity determining region (CDR) H2 sequence
IYPGNGHT

SEQ ID NO: 6 - protein, 13 aa, Artificial Sequence
  Complementarity determining region (CDR) H3 sequence
TRDRANWDDYFDY

SEQ ID NO: 7 - protein, 7 aa, Artificial Sequence
  Complementarity determining region (CDR) H3 sequence
AYDLFNY

SEQ ID NO: 8 - protein, 12 aa, Artificial Sequence
  Complementarity determining region (CDR) L1 sequence
QSLLNSRNQKNH

SEQ ID NO: 9 - protein, 12 aa, Artificial Sequence
  Complementarity determining region (CDR) L1 sequence
QSLLNSDTQKNF

SEQ ID NO: 10 - protein, 9 aa, Artificial Sequence
  Complementarity determining region (CDR) L3 sequence
  MISC_FEATURE (7)..(7): Wherein X is P or no amino acid
QQYYTYXRT

SEQ ID NO: 11 - protein, 9 aa, Artificial Sequence
  Complementarity determining region (CDR) L3 sequence
QQYYSIPLT

SEQ ID NO: 12 - protein, 9 aa, Artificial Sequence
  Complementarity determining region (CDR) H1 sequence
GYSITSDYY

SEQ ID NO: 13 - protein, 8 aa, Artificial Sequence
  Complementarity determining region (CDR) H1 sequence
GYTFTDYY

SEQ ID NO: 14 - protein, 8 aa, Artificial Sequence
  Complementarity determining region (CDR) L3 sequence
QQYYTYRT

SEQ ID NO: 15 - protein, 7 aa, Artificial Sequence
  Complementarity determining region (CDR) H2 sequence
IGYDGSK

SEQ ID NO: 16 - protein, 7 aa, Artificial Sequence
  Complementarity determining region (CDR) H2 sequence
IGYDGTK

SEQ ID NO: 17 - protein, 113 aa, Artificial Sequence
  Sequence from variable light domain (VL)
  MISC_FEATURE (5)..(5): Wherein X is S or T
  MISC_FEATURE (13)..(13): Wherein X is V or M
  MISC_FEATURE (17)..(17): Wherein X is E or O
  MISC_FEATURE (33)..(33): Wherein X is R or D
  MISC_FEATURE (34)..(34): Wherein X is N or T
  MISC_FEATURE (38)..(38): Wherein X is H or F
  MISC_FEATURE (52)..(52): Wherein X is L or I
  MISC_FEATURE (54)..(54): Wherein X is I or V
  MISC_FEATURE (56)..(56): Wherein X is W or F
  MISC_FEATURE (60)..(60): Wherein X is R or K
  MISC_FEATURE (69)..(69): Wherein X is S or I
  MISC_FEATURE (71)..(71): Wherein X is D or S
  MISC_FEATURE (82)..(82): Wherein X is S or T
  MISC_FEATURE (85)..(85): Wherein X is K or Q
  MISC_FEATURE (91)..(91): Wherein X is V or D
  MISC_FEATURE (93)..(93): Wherein X is Y or F
  MISC_FEATURE (99)..(99): Wherein X is T or S
  MISC_FEATURE (100)..(100): Wherein X is Y or I
  MISC_FEATURE (101)..(101): Wherein X is P or no amino acid
  MISC_FEATURE (102)..(102): Wherein X is R or L
  MISC_FEATURE (106)..(106): Wherein X is G or A
DIVMXQSPSSLAXSVGXKVTMSCKSSQSLLNSXXQKNXLAWYQQKPGQSPKXLXYXASTXESGVPDRFXGXGSGTDFTLTIXSVXAEDLAXYXCQQYYXXXXTFGXGTKLEIK

SEQ ID NO: 18 - protein, 112 aa, Artificial Sequence
  Sequence from variable light domain (VL)
  MISC_FEATURE (69)..(69): Wherein X is S or T
DIVMSQSPSSLAVSVGEKVTMSCKSSQSLLNSRNQKNHLAWYQQKPGQSPKLLIYWASTRESGVPDRFXGDGSGTDFTLTISSVKAEDLAVYYCQQYYTYRTFGGGTKLEIK

SEQ ID NO: 19 - protein, 113 aa, Artificial Sequence
  Sequence from variable light domain (VL)
DIVMTQSPSSLAMSVGQKVTMSCKSSQSLLNSDTQKNFLAWYQQKPGQSPKILVYFASTKESGVPDRFIGSGSGTDFTLTITSVQAEDLADYFCQQYYSIPLTFGAGTKLELK

SEQ ID NO: 20 - protein, 120 aa, Artificial Sequence
  Sequence from variable heavy domain (VH)
  MISC_FEATURE (57)..(57): Wherein X is S or T
DVQLQESGPGLVKPSQSLSLTCSVTGYSITSDYYWNWIRQFPGNKLEWMAYIGYDGXKNYNPSLKNRISITRDTSKNQFFLKLNSVTTDDTATYYCTRDRANWDDYFDYWGQGTTLTVSS

SEQ ID NO: 21 - protein, 114 aa, Artificial Sequence
  Sequence from variable heavy domain (VH)
QIQLQQSGPELVKPGAPVKISCKASGYTFTDYYIHWVNQRPGQGLEWIGYIYPGNGHTVYNQKFKVRATLTADNPSSTAYLQLNSLTSEDSGVYFCAYDLFNYWGQGTLVTVSA

SEQ ID NO: 22 - protein, 112 aa, Artificial Sequence
  Sequence of variable light domain (VL)
DIVMSQSPSSLAVSVGEKVTMSCKSSQSLLNSRNQKNHLAWYQQKPGQSPKLLIYWASTRESGVPDRFSGDGSGTDFTLTISSVKAEDLAVYYCQQYYTYRTFGGGTKLEIK

SEQ ID NO: 23 - protein, 112 aa, Artificial Sequence
  Sequence of variable light domain (VL)
DIVMSQSPSSLAVSVGEKVTMSCKSSQSLLNSRNQKNHLAWYQQKPGQSPKLLIYWASTRESGVPDRFTGDGSGTDFTLTISSVKAEDLAVYYCQQYYTYRTFGGGTKLEIK

SEQ ID NO: 24 - protein, 120 aa, Artificial Sequence
  Sequence of variable heavy domain (VH)
DVQLQESGPGLVKPSQSLSLTCSVTGYSITSDYYWNWIRQFPGNKLEWMAYIGYDGSKNYNPSLKNRISITRDTSKNQFFLKLNSVTTDDTATYYCTRDRANWDDYFDYWGQGTTLTVSS

SEQ ID NO: 25 - protein, 120 aa, Artificial Sequence
  Sequence of variable heavy domain (VH)
DVQLQESGPGLVKPSQSLSLTCSVTGYSITSDYYWNWIRQFPGNKLEWMAYIGYDGTKNYNPSLKNRISITRDTSKNQFFLKLNSVTTDDTATYYCTRDRANWDDYFDYWGQGTTLTVSS

SEQ ID NO: 26 - protein, 14 aa, Artificial Sequence
  Antibody, or fragment thereof, binding peptide
GLFGAIAGFIEGGW

SEQ ID NO: 27 - protein, 20 aa, Artificial Sequence
  Signal peptide
MVLQTQVFISLLLWISGAYG

SEQ ID NO: 28 - protein, 19 aa, Artificial Sequence
  Signal peptide
MDWTWRILFLVAAATGTHA

SEQ ID NO: 29 - protein, 469 aa, Artificial Sequence
  Sequence from mAbs
RMKVLSLLYLLTAIPGFLSDVQLQESGPGLVKPSQSLSLTCSVTGYSITSDYYWNWIRQFPGNKLEWMAYIGYDGTKNYNPSLKNRISITRDTSKNQFFLKLNSVTTDDTATYYCTRDRANWDDYFDYWGQGTTLTVSSAKTTAPSVYPLAPVCGDTTGSSVTLGCLVKGYFPEPVTLTWNSGSLSSGVHTFPAVLQSDLYTLSSSVTVTSSTWPSQSITCNVAHPASSTKVDKKIEPRGPTIKPCPPCKCPAPNLLGGPSVFIFPPKIKDVLMISLSPIVTCVVVDVSEDDPDVQISWFVNNVEVHTAQTQTHREDYNSTLRVVSALPIQHQDWMSGKEFKCKVNNKDLPAPIERTISKPKGSVRAPQVYVLPPPEEEMTKKQVTLTCMVTDFMPEDIYVEWTNNGKTELNYKNTEPVLDSDGSYFMYSKLRVEKKNWVERNSYSCSVVHEGLHNHHTTKSFSRTPGK

SEQ ID NO: 30 - protein, 233 aa, Artificial Sequence
  Sequence from mAbs
VLMLLLLWVSGTCGDIVMSQSPSSLAVSVGEKVTMSCKSSQSLLNSRNQKNHLAWYQQKPGQSPKLLIYWASTRESGVPDRFTGDGSGTDFTLTISSVKAEDLAVYYCQQYYTYRTFGGGTKLEIKRADAAPTVSIFPPSSEQLTSGGASVVCFLNNFYPKDINVKWKIDGSERQNGVLNSWTDQDSKDSTYSMSSTLTLTKDEYERHNSYTCEATHKTSTSPIVKSFNRNEC

SEQ ID NO: 31 - protein, 449 aa, Artificial Sequence
  Sequence from mAbs
AGVHCQIQLQQSGPELVKPGAPVKISCKASGYTFTDYYIHWVNQRPGQGLEWIGYIYPGNGHTVYNQKFKVRATLTADNPSSTAYLQLNSLTSEDSGVYFCAYDLFNYWGQGTLVTVSAAKTTAPSVYPLAPVCGDTTGSSVTLGCLVKGYFPEPVTLTWNSGSLSSGVHTFPAVLQSDLYTLSSSVTVTSSTWPSQSITCNVAHPASSTKVDKKIEPRGPTIKPCPPCKCPAPNLLGGPSVFIFPPKIKDVLMISLSPIVTCVVVDVSEDDPDVQISWFVNNVEVHTAQTQTHREDYNSTLRVVSALPIQHQDWMSGKEFKCKVNNKDLPAPIERTISKPKGSVRAPQVYVLPPPEEEMTKKQVTLTCMVTDFMPEDIYVEWTNNGKTELNYKNTEPVLDSDGSYFMYSKLRVEKKNWVERNSYSCSVVHEGLHNHHTTKSFSRTPGK

SEQ ID NO: 32 - protein, 226 aa, Artificial Sequence
  Sequence from mAbs
VSGACADIVMTQSPSSLAMSVGQKVTMSCKSSQSLLNSDTQKNFLAWYQQKPGQSPKILVYFASTKESGVPDRFIGSGSGTDFTLTITSVQAEDLADYFCQQYYSIPLTFGAGTKLELKRADAAPTVSIFPPSSEQLTSGGASVVCFLNNFYPKDINVKWKIDGSERQNGVLNSWTDQDSKDSTYSMSSTLTLTKDEYERHNSYTCEATHKTSTSPIVKSFNRNEC

SEQ ID NO: 33 - protein, 469 aa, Artificial Sequence
  Sequence from mAbs
RMKVLSLLYLLTAIPGFLSDVQLQESGPGLVKPSQSLSLTCSVTGYSITSDYYWNWIRQFPGNKLEWMAYIGYDGSKNYNPSLKNRISITRDTSKNQFFLKLNSVTTDDTATYYCTRDRANWDDYFDYWGQGTTLTVSSAKTTAPSVYPLAPVCGDTTGSSVTLGCLVKGYFPEPVTLTWNSGSLSSGVHTFPAVLQSDLYTLSSSVTVTSSTWPSQSITCNVAHPASSTKVDKKIEPRGPTIKPCPPCKCPAPNLLGGPSVFIFPPKIKDVLMISLSPIVTCVVVDVSEDDPDVQISWFVNNVEVHTAQTQTHREDYNSTLRVVSALPIQHQDWMSGKEFKCKVNNKDLPAPIERTISKPKGSVRAPQVYVLPPPEEEMTKKQVTLTCMVTDFMPEDIYVEWTNNGKTELNYKNTEPVLDSDGSYFMYSKLRVEKKNWVERNSYSCSVVHEGLHNHHTTKSFSRTPGK

SEQ ID NO: 34 - protein, 233 aa, Artificial Sequence
  Sequence from mAbs
VLMLLLLWVSGTCGDIVMSQSPSSLAVSVGEKVTMSCKSSQSLLNSRNQKNHLAWYQQKPGQSPKLLIYWASTRESGVPDRFSGDGSGTDFTLTISSVKAEDLAVYYCQQYYTYRTFGGGTKLEIKRADAAPTVSIFPPSSEQLTSGGASVVCFLNNFYPKDINVKWKIDGSERQNGVLNSWTDQDSKDSTYSMSSTLTLTKDEYERHNSYTCEATHKTSTSPIVKSFNRNEC

SEQ ID NO: 35 - protein, 731 aa, Artificial Sequence
  mAb 10A9 sequence
METDTLLLWVLLLWVPGSTGQIQLQQSGPELVKPGAPVKISCKASGYTFTDYYIHWVNQRPGQGLEWIGYIYPGNGHTVYNQKFKVRATLTADNPSSTAYLQLNSLTSEDSGVYFCAYDLFNYWGQGTLVTVSAAKTTAPSVYPLAPVCGDTTGSSVTLGCLVKGYFPEPVTLTWNSGSLSSGVHTFPAVLQSDLYTLSSSVTVTSSTWPSQSITCNVAHPASSTKVDKKIEPRGPTIKPCPPCKCPAPNLLGGPSVFIFPPKIKDVLMISLSPIVTCVVVDVSEDDPDVQISWFVNNVEVHTAQTQTHREDYNSTLRVVSALPIQHQDWMSGKEFKCKVNNKDLPAPIERTISKPKGSVRAPQVYVLPPPEEEMTKKQVTLTCMVTDFMPEDIYVEWTNNGKTELNYKNTEPVLDSDGSYFMYSKLRVEKKNWVERNSYSCSVVHEGLHNHHTTKSFSRTPGRKRRAPVKQTLNFDLLKLAGDVESNPGPMETDTLLLWVLLLWVPGSTGDIVMTQSPSSLAMSVGQKVTMSCKSSQSLLNSDTQKNFLAWYQQKPGQSPKILVYFASTKESGVPDRFIGSGSGTDFTLTITSVQAEDLADYFCQQYYSIPLTFGAGTKLELKRADAAPTVSIFPPSSEQLTSGGASVVCFLNNFYPKDINVKWKIDGSERQNGVLNSWTDQDSKDSTYSMSSTLTLTKDEYERHNSYTCEATHKTSTSPIVKSFNRNEC

SEQ ID NO: 36 - protein, 736 aa, Artificial Sequence
  mAb 11H12 sequence
METDTLLLWVLLLWVPGSTGDVQLQESGPGLVKPSQSLSLTCSVTGYSITSDYYWNWIRQFPGNKLEWMAYIGYDGTKNYNPSLKNRISITRDTSKNQFFLKLNSVTTDDTATYYCTRDRANWDDYFDYWGQGTTLTVSSAKTTAPSVYPLAPVCGDTTGSSVTLGCLVKGYFPEPVTLTWNSGSLSSGVHTFPAVLQSDLYTLSSSVTVTSSTWPSQSITCNVAHPASSTKVDKKIEPRGPTIKPCPPCKCPAPNLLGGPSVFIFPPKIKDVLMISLSPIVTCVVVDVSEDDPDVQISWFVNNVEVHTAQTQTHREDYNSTLRVVSALPIQHQDWMSGKEFKCKVNNKDLPAPIERTISKPKGSVRAPQVYVLPPPEEEMTKKQVTLTCMVTDFMPEDIYVEWTNNGKTELNYKNTEPVLDSDGSYFMYSKLRVEKKNWVERNSYSCSVVHEGLHNHHTTKSFSRTPGRKRRAPVKQTLNFDLLKLAGDVESNPGPMETDTLLLWVLLLWVPGSTGDIVMSQSPSSLAVSVGEKVTMSCKSSQSLLNSRNQKNHLAWYQQKPGQSPKLLIYWASTRESGVPDRFTGDGSGTDFTLTISSVKAEDLAVYYCQQYYTYRTFGGGTKLEIKRADAAPTVSIFPPSSEQLTSGGASVVCFLNNFYPKDINVKWKIDGSERQNGVLNSWTDQDSKDSTYSMSSTLTLTKDEYERHNSYTCEATHKTSTSPIVKSFNRNEC